European Patent Application EP 4 778 510 A1, published July 22, 2026. Title: SKIN CARE COMPOSITION AND USES THEREOF. Applicant: S-BIOMEDIC NV. Application EP. The sequence listing filed with the application follows.

SEQUENCE LISTING (7 sequences)

SEQ ID NO: 1 - DNA, 21 bp, synthetic construct
  source 1..21: mol_type = other DNA
cagcggcgctgctaagaactt

SEQ ID NO: 2 - DNA, 20 bp, synthetic construct
  source 1..20: mol_type = other DNA
ccggctggcaaatgaggcat

SEQ ID NO: 3 - DNA, 54 bp, synthetic construct
  source 1..54: mol_type = other DNA
tcgtcggcagcgtcagatgtgtataagagacagcagcggcgctgctaagaactt

SEQ ID NO: 4 - DNA, 54 bp, synthetic construct
  source 1..54: mol_type = other DNA
gtctcgtgggctcggagatgtgtataagagacagccggctggcaaatgaggcat

SEQ ID NO: 5 - DNA, 484 bp, Propionibacterium acnes
  source 1..484: mol_type = genomic DNA
gttgcacaccagggggtcaacttggcgtcctcagttcaaaattgattcaaactaacagttccatgtcgggaaacagcaccaggaagctcgtgacatatcgtctttcattgcgagaaacatcttacttatgtacatttctaagctatagcgtctacccttgtcagacccaggacgatgggtgtcacatctcctttctagtcaacctaagagaggaggaaatgccgcgatatatgttccaccctgtcatcacgaaggccaccacaatctatcccagaacagccggcacttcactcacgatgccccgatgctggattcctattgtcgcccttattagggcaagcggtgccagtagcagaatatgtcacctcaacaactcgatccacccctgcccattacatgggtaacatatccatggaggttcgatgtatactcgaggatacagtcgtccatcacgcccgcctacatacccattacatcagcatag

SEQ ID NO: 6 - DNA, 484 bp, Propionibacterium acnes
  source 1..484: mol_type = genomic DNA
gttgcacaccagggggtcaacttggcgtcctcagttcaaaattgattcaaactaacagttccatgtcgggaaacagcaccaggaaactcgtgacatatcgtctttcattgcgagaaacatcttacttatgtacatttctaagctatagcgtctacccttgtcagacccaggacgatgggtgtcacatcccctttctagtcaacctaagagaggaggaaatgccgcgatatatgttccgccctgtcatcacgaagaccaccacaatctatcccagaacagccggcacttcactcacgatgccccgatgctggattcctattgtcgcccttattagggcaagcggtgccagtagcagaatatgtcacctcaacaactcgatccacccctgcccattacatgggtaacatatccatggaggttcgatgtatacttgaggatacagtcgtccatcacgcccacctacatacccattacatcagcatag

SEQ ID NO: 7 - DNA, 484 bp, Propionibacterium acnes
  source 1..484: mol_type = genomic DNA
gttgcacaccagggggtcaacttggcgtcctcagttcaaaattgattcaaactaacagttccatgtcgggaaacagcaccaggaagctcgtgacatatcgtctttcattgcgagaaacatcttacttatgtacatttctaagctatatcgtctacccttgtcagacccaggacgatggatgtcacatcccctttctagtcaacctaagagaggaggaaatgccgcgatatatgttccaccctgtcatcacgaaggccaccacaatctatcccagaacagccggcacttcactcacgatgccccgatgctggattcctattgtcgcccttattagggcaagcggtgccagtagcagaatatgtcacctcaacaactcgatccacccctgcccattacatgggtaacatatccatggaggttcgatgtatattcgaggatacagtcgtccatcacgcccgcctacatacccattacatcagcatag